European Patent Specification EP 3 870 224 B1, published July 8, 2026. Title: METHODS AND COMPOSITIONS. Applicant: United Kingdom Research and Innovation. Application PCT/GB2019/053023. The sequence listing filed with the application follows.

SEQUENCE LISTING (38 sequences)

SEQ ID NO: 1 - DNA, 72 bp, Methanosarcina barkeri
gggaacctgatcatgtagatcgaatggactctaaatccgttcagccgggttagattcccggggtttccgcca

SEQ ID NO: 2 - DNA, 72 bp, Methanosarcina barkeri
ggaaacctgatcatgtagatcgaatggactctaaatccgttcagccgggttagattcccggggtttccgcca

SEQ ID NO: 3 - protein, 419 aa, Artificial Sequence
  DAPRS synthetase
MDKKPLDVLISATGLWMSRTGTLHKIKHHEVSRSKIYIEMACGDHLVVNNSRSCRTARAFRHHKYRKTCKRCRVSDEDINNFLTRSTESKNSVKVRVVSAPKVKKAMPKSVSRAPKPLENSVSAKASTNTSRSVPSPAKSTPNSSVPASAPAPSLTRSQLDRVEALLSPEDKISLNMAKPFRELEPELVTRRKNDFQRLYTNDREDYLGKLERDITKFFVDRGFLEIKSPILIPAEYVERMGINNDTELSKQIFRVDKNLCLRPMLAPTLCNYLRKLDRILPGPIKIFEVGPCYRKESDGKEHLEEFTMVQFCQMGSGCTRENLEALIKEFLDYLEIDFEIVGDSCMVFGDTLDIMHGDLELSSACVGPVSLDREWGIDKPWIGAGFGLERLLKVMHGFKNIKRASRSESYYNGISTNL

SEQ ID NO: 4 - protein, 419 aa, Methanosarcina barkeri
MDKKPLDVLISATGLWMSRTGTLHKIKHHEVSRSKIYIEMACGDHLVVNNSRSCRTARAFRHHKYRKTCKRCRVSDEDINNFLTRSTESKNSVKVRVVSAPKVKKAMPKSVSRAPKPLENSVSAKASTNTSRSVPSPAKSTPNSSVPASAPAPSLTRSQLDRVEALLSPEDKISLNMAKPFRELEPELVTRRKNDFQRLYTNDREDYLGKLERDITKFFVDRGFLEIKSPILIPAEYVERMGINNDTELSKQIFRVDKNLCLRPMLAPTLYNYLRKLDRILPGPIKIFEVGPCYRKESDGKEHLEEFTMVNFCQMGSGCTRENLEALIKEFLDYLEIDFEIVGDSCMVYGDTLDIMHGDLELSSAVVGPVSLDREWGIDKPWIGAGFGLERLLKVMHGFKNIKRASRSESYYNGISTNL

SEQ ID NO: 5 - protein, 419 aa, Methanosarcina barkeri
MDKKPLDVLISATGLWMSRTGTLHKIKHYEVSRSKIYIEMACGDHLVVNNSRSCRTARAFRHHKYRKTCKRCRVSDEDINNFLTRSTEGKTSVKVKVVSAPKVKKAMPKSVSRAPKPLENPVSAKASTDTSRSVPSPAKSTPNSPVPTSAPAPSLTRSQLDRVEALLSPEDKISLNIAKPFRELESELVTRRKNDFQRLYTNDREDYLGKLERDITKFFVDRDFLEIKSPILIPAEYVERMGINNDTELSKQIFRVDKNLCLRPMLAPTLYNYLRKLDRILPDPIKIFEVGPCYRKESDGKEHLEEFTMVNFCQMGSGCTRENLESLIKEFLDYLEIDFEIVGDSCMVYGDTLDIMHGDLELSSAVVGPVPLDREWGIDKPWIGAGFGLERLLKVMHGFKNIKRASRSESYYNGISTNL

SEQ ID NO: 6 - protein, 454 aa, Methanosarcina mazeii
MDKKPLNTLISATGLWMSRTGTIHKIKHHEVSRSKIYIEMACGDHLVVNNSRSSRTARALRHHKYRKTCKRCRVSDEDLNKFLTKANEDQTSVKVKVVSAPTRTKKAMPKSVARAPKPLENTEAAQAQPSGSKFSPAIPVSTQESVSVPASVSTSISSISTGATASALVKGNTNPITSMSAPVQASAPALTKSQTDRLEVLLNPKDEISLNSGKPFRELESELLSRRKKDLQQIYAEERENYLGKLEREITRFFVDRGFLEIKSPILIPLEYIERMGIDNDTELSKQIFRVDKNFCLRPMLAPNLYNYLRKLDRALPDPIKIFEIGPCYRKESDGKEHLEEFTMLNFCQMGSGCTRENLESIITDFLNHLGIDFKIVGDSCMVYGDTLDVMHGDLELSSAVVGPIPLDREWGIDKPWIGAGFGLERLLKVKHDFKNIKRAARSESYYNGISTNL

SEQ ID NO: 7 - protein, 443 aa, Methanosarcina acetivorans
MDKKPLDTLISATGLWMSRTGMIHKIKHHEVSRSKIYIEMACGERLVVNNSRSSRTARALRHHKYRKTCRHCRVSDEDINNFLTKTSEEKTTVKVKVVSAPRVRKAMPKSVARAPKPLEATAQVPLSGSKPAPATPVSAPAQAPAPSTGSASATSASAQRMANSAAAPAAPVPTSAPALTKGQLDRLEGLLSPKDEISLDSEKPFRELESELLSRRKKDLKRIYAEERENYLGKLEREITKFFVDRGFLEIKSPILIPAEYVERMGINSDTELSKQVFRIDKNFCLRPMLAPNLYNYLRKLDRALPDPIKIFEIGPCYRKESDGKEHLEEFTMLNFCQMGSGCTRENLEAIITEFLNHLGIDFEIIGDSCMVYGNTLDVMHDDLELSSAVVGPVPLDREWGIDKPWIGAGFGLERLLKVMHGFKNIKRAARSESYYNGISTNL

SEQ ID NO: 8 - protein, 478 aa, Methanosarcina thermophila
MDKKPLNTLISATGLWMSRTGKLHKIRHHEVSKRKIYIEMECGERLVVNNSRSCRAARALRHHKYRKICKHCRVSDEDLNKFLTRTNEDKSNAKVTVVSAPKIRKVMPKSVARTPKPLENTAPVQTLPSESQPAPTTPISASTTAPASTSTTAPAPASTTAPAPASTTAPASASTTISTSAMPASTSAQGTTKFNYISGGFPRPIPVQASAPALTKSQIDRLQGLLSPKDEISLDSGTPFRKLESELLSRRRKDLKQIYAEEREHYLGKLEREITKFFVDRGFLEIKSPILIPMEYIERMGIDNDKELSKQIFRVDNNFCLRPMLAPNLYNYLRKLNRALPDPIKIFEIGPCYRKESDGKEHLEEFTMLNFCQMGSGCTRENLEAIIKDFLDYLGIDFEIVGDSCMVYGDTLDVMHGDLELSSAVVGPVPMDRDWGINKPWIGAGFGLERLLKVMHNFKNIKRASRSESYYNGISTNL

SEQ ID NO: 9 - protein, 416 aa, Methanococcoides burtonii
MEKQLLDVLVELNGVWLSRSGLLHGIRNFEITTKHIHIETDCGARFTVRNSRSSRSARSLRHNKYRKPCKRCRPADEQIDRFVKKTFKEKRQTVSVFSSPKKHVPKKPKVAVIKSFSISTPSPKEASVSNSIPTPSISVVKDEVKVPEVKYTPSQIERLKTLMSPDDKIPIQDELPEFKVLEKELIQRRRDDLKKMYEEDREDRLGKLERDITEFFVDRGFLEIKSPIMIPFEYIERMGIDKDDHLNKQIFRVDESMCLRPMLAPCLYNYLRKLDKVLPDPIRIFEIGPCYRKESDGSSHLEEFTMVNFCQMGSGCTRENMEALIDEFLEHLGIEYEIEADNCMVYGDTIDIMHGDLELSSAVVGPIPLDREWGVNKPWMGAGFGLERLLKVRHNYTNIRRASRSELYYNGINTNL

SEQ ID NO: 10 - protein, 279 aa, Desulfitobacterium hafniense
MSSFWTKVQYQRLKELNASGEQLEMGFSDALSRDRAFQGIEHQLMSQGKRHLEQLRTVKHRPALLELEEGLAKALHQQGFVQVVTPTIITKSALAKMTIGEDHPLFSQVFWLDGKKCLRPMLAPNLYTLWRELERLWDKPIRIFEIGTCYRKESQGAQHLNEFTMLNLTELGTPLEERHQRLEDMARWVLEAAGIREFELVTESSVVYGDTVDVMKGDLELASGAMGPHFLDEKWEIVDPWVGLGFGLERLLMIREGTQHVQSMARSLSYLDGVRLNIN

SEQ ID NO: 11 - protein, 312 aa, Desulfitobacterium hafniense
MDRIDHTDSKFVQAGETPVLPATFMFLTRRDPPLSSFWTKVQYQRLKELNASGEQLEMGFSDALSRDRAFQGIEHQLMSQGKRHLEQLRTVKHRPALLELEEGLAKALHQQGFVQVVTPTIITKSALAKMTIGEDHPLFSQVFWLDGKKCLRPMLAPNLYTLWRELERLWDKPIRIFEIGTCYRKESQGAQHLNEFTMLNLTELGTPLEERHQRLEDMARWVLEAAGIREFELVTESSVVYGDTVDVMKGDLELASGAMGPHFLDEKWEIVDPWVGLGFGLERLLMIREGTQHVQSMARSLSYLDGVRLNIN

SEQ ID NO: 12 - protein, 288 aa, Desulfitobacterium hafniense
MFLTRRDPPLSSFWTKVQYQRLKELNASGEQLEMGFSDALSRDRAFQGIEHQLMSQGKRHLEQLRTVKHRPALLELEEKLAKALHQQGFVQVVTPTIITKSALAKMTIGEDHPLFSQVFWLDGKKCLRPMLAPNLYTLWRELERLWDKPIRIFEIGTCYRKESQGAQHLNEFTMLNLTELGTPLEERHQRLEDMARWVLEAAGIREFELVTESSVVYGDTVDVMKGDLELASGAMGPHFLDEKWEIFDPWVGLGFGLERLLMIREGTQHVQSMARSLSYLDGVRLNIN

SEQ ID NO: 13 - protein, 277 aa, Desulfotomaculum acetoxidans
MSFLWTVSQQKRLSELNASEEEKNMSFSSTSDREAAYKRVEMRLINESKQRLNKLRHETRPAICALENRLAAALRGAGFVQVATPVILSKKLLGKMTITDEHALFSQVFWIEENKCLRPMLAPNLYYILKDLLRLWEKPVRIFEIGSCFRKESQGSNHLNEFTMLNLVEWGLPEEQRQKRISELAKLVMDETGIDEYHLEHAESVVYGETVDVMHRDIELGSGALGPHFLDGRWGVVGPWVGIGFGLERLLMVEQGGQNVRSMGKSLTYLDGVRLNI

SEQ ID NO: 14 - protein, 419 aa, Methanosarcina barkeri; identical to SEQ ID NO: 5

SEQ ID NO: 15 - protein, 419 aa, Artificial Sequence; identical to SEQ ID NO: 4
  artificial synthetase

SEQ ID NO: 16 - protein, 419 aa, Artificial Sequence
  AcKRS synthetase
MDKKPLDVLISATGLWMSRTGTLHKIKHHEVSRSKIYIEMACGDHLVVNNSRSCRTARAFRHHKYRKTCKRCRVSGEDINNFLTRSTESKNSVKVRVVSAPKVKKAMPKSVSRAPKPLENSVSAKASTNTSRSVPSPAKSTPNSSVPASAPAPSLTRSQLDRVEALLSPEDKISLNMAKPFRELEPELVTRRKNDFQRLYTNDREDYLGKLERDITKFFVDRGFLEIKSPILIPAEYVERMGINNDTELSKQIFRVDKNLCLRPMVAPTIFNYARKLDRILPGPIKIFEVGPCYRKESDGKEHLEEFTMVNFFQMGSGCTRENLEALIKEFLDYLEIDFEIVGDSCMVYGDTLDIMHGDLELSSAVVGPVSLDREWGIDKPWIGAGFGLERLLKVMHGFKNIKRASRSESYYNGISTNL

SEQ ID NO: 17 - protein, 419 aa, Artificial Sequence
  PCKRS synthetase
MDKKPLDVLISATGLWMSRTGTLHKIKHHEVSRSKIYIEMACGDHLVVNNSRSCRTARAFRHHKYRKTCKRCRVSDEDINNFLTRSTESKNSVKVRVVSAPKVKKAMPKSVSRAPKPLENSVSAKASTNTSRSVPSPAKSTPNSSVPASAPAPSLTRSQLDRVEALLSPEDKISLNMAKPFRELEPELVTRRKNDFQRLYTNDREDYLGKLERDITKFFVDRGFLEIKSPILIPAEYVERFGINNDTELSKQIFRVDKNLCLRPMLSPTLCNYMRKLDRILPGPIKIFEVGPCYRKESDGKEHLEEFTMVNFCQMGSGCTRENLEALIKEFLDYLEIDFEIVGDSCMVYGDTLDIMHGDLELSSAVVGPVSLDREWGIDKPWIGAGFGLERLLKVMHGFKNIKRASRSESYYNGISTNL

SEQ ID NO: 18 - protein, 454 aa, Artificial Sequence; identical to SEQ ID NO: 6
  artificial synthetase

SEQ ID NO: 19 - protein, 454 aa, Artificial Sequence
  Mm-ACKRS synthetase
MDKKPLNTLISATGLWMSRTGTIHKIKHHEVSRSKIYIEMACGDHLVVNNSRSSRTARALRHHKYRKTCKRCRVSDEDLNKFLTKANEDQTSVKVKVVSAPTRTKKAMPKSVARAPKPLENTEAAQAQPSGSKFSPAIPVSTQESVSVPASVSTSISSISTGATASALVKGNTNPITSMSAPVQASAPALTKSQTDRLEVLLNPKDEISLNSGKPFRELESELLSRRKKDLQQIYAEERENYLGKLEREITRFFVDRGFLEIKSPILIPLEYIERMGIDNDTELSKQIFRVDKNFCLRPMVAPNIFNYARKLDRALPDPIKIFEIGPCYRKESDGKEHLEEFTMLNFFQMGSGCTRENLESIITDFLNHLGIDFKIVGDSCMVYGDTLDVMHGDLELSSAVVGPIPLDREWGIDKPWIGAGFGLERLLKVKHDFKNIKRAARSESYYNGISTNL

SEQ ID NO: 20 - protein, 454 aa, Artificial Sequence
  Mm-PCKRS synthetase
MDKKPLNTLISATGLWMSRTGTIHKIKHHEVSRSKIYIEMACGDHLVVNNSRSSRTARALRHHKYRKTCKRCRVSDEDLNKFLTKANEDQTSVKVKVVSAPTRTKKAMPKSVARAPKPLENTEAAQAQPSGSKFSPAIPVSTQESVSVPASVSTSISSISTGATASALVKGNTNPITSMSAPVQASAPALTKSQTDRLEVLLNPKDEISLNSGKPFRELESELLSRRKKDLQQIYAEERENYLGKLEREITRFFVDRGFLEIKSPILIPLEYIERFGIDNDTELSKQIFRVDKNFCLRPMLSPNLCNYMRKLDRALPDPIKIFEIGPCYRKESDGKEHLEEFTMLNFCQMGSGCTRENLESIITDFLNHLGIDFKIVGDSCMVYGDTLDVMHGDLELSSAVVGPIPLDREWGIDKPWIGAGFGLERLLKVKHDFKNIKRAARSESYYNGISTNL

SEQ ID NO: 21 - DNA, 49 bp, Artificial Sequence
  primer
  misc_feature (19)..(20): n is a, c, g, or t
ggaaaggtctcgaccctgnnkaactatctgcgtaaactggatcgtattc

SEQ ID NO: 22 - DNA, 37 bp, Artificial Sequence
  primer
ggaaaggtctcagggtcggggccagcatcggacgcag

SEQ ID NO: 23 - DNA, 48 bp, Artificial Sequence
  primer
  misc_feature (19)..(20): n is a, c, g, or t
ggaaaggtctccatggttnnkttttgccaaatgggcagcggctgcacc

SEQ ID NO: 24 - DNA, 42 bp, Artificial Sequence
  primer
ggaaaggtctcaccatggtgaattcttccaggtgttctttgc

SEQ ID NO: 25 - DNA, 47 bp, Artificial Sequence
  primer
  misc_feature (19)..(20): n is a, c, g, or t
ggaaaggtctccatggtgnnkggcgataccctggatattatgcatgg

SEQ ID NO: 26 - DNA, 43 bp, Artificial Sequence
  primer
ggaaaggtctcaccatgcagctatcgcccacaatttcgaagtc

SEQ ID NO: 27 - DNA, 46 bp, Artificial Sequence
  primer
  misc_feature (19)..(20): n is a, c, g, or t
ggaaaggtctccagcgcgnnkgtgggtccggttagcctggatcgtg

SEQ ID NO: 28 - DNA, 38 bp, Artificial Sequence
  primer
ggaaaggtctcgcgctgctcagttccagatcgccatgc

SEQ ID NO: 29 - DNA, 47 bp, Artificial Sequence
  primer
  misc_feature (19)..(20): n is a, c, g, or t
ggaaaggtctctaaaccgnnkattggcgcgggttttggcctggaacg

SEQ ID NO: 30 - DNA, 38 bp, Artificial Sequence
  primer
ggaaaggtctcggtttatcaatgccccattcacgatcc

SEQ ID NO: 31 - DNA, 44 bp, Artificial Sequence
  primer
ggaaaggtctcgtagggcagtccattagtatcaactagagatgg

SEQ ID NO: 32 - DNA, 44 bp, Artificial Sequence
  primer
ggaaaggtctcccctactgcccatccttggtttgaatccaatgc

SEQ ID NO: 33 - DNA, 44 bp, Artificial Sequence
  primer
ggaaaggtctcggctggcagtccattagtatcaactagagatgg

SEQ ID NO: 34 - DNA, 44 bp, Artificial Sequence
  primer
ggaaaggtctcccagcctgcccatccttggtttgaatccaatgc

SEQ ID NO: 35 - DNA, 31 bp, Artificial Sequence
  primer
ttattacatatgcatcatcatcaccaccatc

SEQ ID NO: 36 - DNA, 24 bp, Artificial Sequence
  primer
ataataactcgagttagccacgcg

SEQ ID NO: 37 - DNA, 35 bp, Artificial Sequence
  primer
gtgtatatcggtggtcactagctgggtggccatat

SEQ ID NO: 38 - DNA, 35 bp, Artificial Sequence
  primer
atatggccacccagctagtgaccaccgatatacac